European Patent Application EP 4 814 011 A1, published September 30, 2026. Title: 靶向TSLP的抗原结合蛋白及应用. Applicant: 上海华奥泰生物药业股份有限公司. The sequence listing filed with the application follows.

SEQUENCE LISTING (48 sequences)

SEQ ID NO: 1 - protein, 8 aa, synthetic construct
  REGION 1..8: note = HCDR1 of 900792 900792VH1 900792VH2 900792VH3 900792VH4
GYAFTNYL

SEQ ID NO: 2 - protein, 8 aa, synthetic construct
  REGION 1..8: note = HCDR2 of 900792 900792VH1 900792VH2 900792VH3 900792VH4
INPESGDT

SEQ ID NO: 3 - protein, 12 aa, synthetic construct
  REGION 1..12: note = HCDR3 of 900792 900792VH1 900792VH2 900792VH3 900792VH4
AKESLTGSSYDY

SEQ ID NO: 4 - protein, 6 aa, synthetic construct
  REGION 1..6: note = LCDR1 of 900792 900792VL1 900792VL2 900792VL3
ENIYSN

SEQ ID NO: 5 - skipped

SEQ ID NO: 6 - protein, 9 aa, synthetic construct
  REGION 1..9: note = LCDR3 of 900792 900792VL1 900792VL2 900792VL3
QHFYETPLT

SEQ ID NO: 7 - protein, 25 aa, synthetic construct
  REGION 1..25: note = FR1-900792-VH
QVQLQQSGAELVRPGTSVLVSCKAS

SEQ ID NO: 8 - protein, 25 aa, synthetic construct
  REGION 1..25: note = FR1-900792-VH1 FR1-900792-VH3
QVQLQQSGAEVKKPGASVKVSCKAS

SEQ ID NO: 9 - protein, 25 aa, synthetic construct [sequence omitted]

SEQ ID NO: 10 - protein, 17 aa, synthetic construct
  REGION 1..17: note = FR2-900792-VH
IEWVLQRPGQGLEWIGV

SEQ ID NO: 11 - protein, 17 aa, synthetic construct
  REGION 1..17: note = FR2-900792-VH1
IEWVRQAPGQGLEWIGV

SEQ ID NO: 12 - protein, 17 aa, synthetic construct
  REGION 1..17: note = FR2-900792-VH2 FR2-900792-VH4
IEWVRQAPGQGLEWMGI

SEQ ID NO: 13 - protein, 17 aa, synthetic construct
  REGION 1..17: note = FR2-900792-VH3
IEWVRQAPGQGLEWMGV

SEQ ID NO: 14 - protein, 37 aa, synthetic construct
  REGION 1..37: note = FR3-900792-VH
YSEKFKGKATLTADKSSSTAYMQLSSLTSEDSAVYFC

SEQ ID NO: 15 - protein, 38 aa, synthetic construct
  REGION 1..38: note = FR3-900792-VH1
YYSEKFQGRVTLTADKSTSTAYMELSSLRSEDSAVYFC

SEQ ID NO: 16 - protein, 38 aa, synthetic construct
  REGION 1..38: note = FR3-900792-VH2
YYAQKFQGRVTMTADKSTSTAYMELSSLRSEDSAVYFC

SEQ ID NO: 17 - protein, 38 aa, synthetic construct
  REGION 1..38: note = FR3-900792-VH3
YYSQKFQGRVTMTADKSTSTAYMELSSLRSEDSAVYFC

SEQ ID NO: 18 - protein, 38 aa, synthetic construct
  REGION 1..38: note = FR3-900792-VH4
YYAQKFQGRVTLTADKSTSTAYMELSSLRSEDSAVYYC

SEQ ID NO: 19 - protein, 11 aa, synthetic construct
  REGION 1..11: note = FR4-900792-VH
WGQGTTLTVSS

SEQ ID NO: 20 - protein, 13 aa, synthetic construct
  REGION 1..13: note = FR4-900792-VH1 FR4-900792-VH2 FR4-900792-VH3 FR4-900792-VH4
DYWGQGTTLTVSS

SEQ ID NO: 21 - protein, 26 aa, synthetic construct
  REGION 1..26: note = FR1-900792-VL
DIQMTQSPASLSASVGESVTITCRAS

SEQ ID NO: 22 - protein, 26 aa, synthetic construct [sequence omitted]

SEQ ID NO: 23 - protein, 17 aa, synthetic construct
  REGION 1..17: note = FR2-900792-VL
LVWYQQKQGKSPQLLVY

SEQ ID NO: 24 - protein, 17 aa, synthetic construct
  REGION 1..17: note = FR2-900792-VL1 FR2-900792-VL2
LVWYQQKPGKAPQLLVY

SEQ ID NO: 25 - protein, 17 aa, synthetic construct
  REGION 1..17: note = FR2-900792-VL3
LVWYQQKPGKAPQLLIY

SEQ ID NO: 26 - protein, 36 aa, synthetic construct
  REGION 1..36: note = FR3-900792-VL
NLADGVPSRFSGSGSGTQFSLKINSLQPEDFGNYYC

SEQ ID NO: 27 - protein, 36 aa, synthetic construct
  REGION 1..36: note = FR3-900792-VL1
NLADGVPSRFSGSGSGTQFSLTISSLQPEDFATYYC

SEQ ID NO: 28 - protein, 36 aa, synthetic construct
  REGION 1..36: note = FR3-900792-VL2
NLQSGVPSRFSGSGSGTQFSLTISSLQPEDFATYYC

SEQ ID NO: 29 - protein, 36 aa, synthetic construct
  REGION 1..36: note = FR3-900792-VL3
NLQSGVPSRFSGSGSGTQFTLTISSLQPEDFATYYC

SEQ ID NO: 30 - protein, 10 aa, synthetic construct
  REGION 1..10: note = FR4-900792-VL1 FR4-900792-VL2 FR4-900792-VL3
FGTGTKLEIK

SEQ ID NO: 31 - protein, 119 aa, synthetic construct
  REGION 1..119: note = 900792-VH
QVQLQQSGAELVRPGTSVKVSCKASGYAFTNYLIEWVKQRPGQGLEWIGVINPESGDTYYSEKFKGKATLTADKSSSTAYMQLSSLTSEDSAVYFCAKESLTGSSYDYWGQGTTLTVSS

SEQ ID NO: 32 - protein, 119 aa, synthetic construct
  REGION 1..119: note = 900792-VH1
QVQLQQSGAEVKKPGASVKVSCKASGYAFTNYLIEWVRQAPGQGLEWIGVINPESGDTYYSEKFQGRVTLTADKSTSTAYMELSSLRSEDSAVYFCAKESLTGSSYDYWGQGTTLTVSS

SEQ ID NO: 33 - protein, 119 aa, synthetic construct
  REGION 1..119: note = 900792-VH2
QVQLVQSGAEVKKPGASVKVSCKASGYAFTNYLIEWVRQAPGQGLEWMGIINPESGDTYYAQKFQGRVTMTADKSTSTAYMELSSLRSEDSAVYFCAKESLTGSSYDYWGQGTTLTVSS

SEQ ID NO: 34 - protein, 119 aa, synthetic construct
  REGION 1..119: note = 900792-VH3
QVQLQQSGAEVKKPGASVKVSCKASGYAFTNYLIEWVRQAPGQGLEWMGVINPESGDTYYSQKFQGRVTMTADKSTSTAYMELSSLRSEDSAVYFCAKESLTGSSYDYWGQGTTLTVSS

SEQ ID NO: 35 - protein, 119 aa, synthetic construct
  REGION 1..119: note = 900792-VH4
QVQLVQSGAEVKKPGASVKVSCKASGYAFTNYLIEWVRQAPGQGLEWMGIINPESGDTYYAQKFQGRVTLTADKSTSTAYMELSSLRSEDSAVYYCAKESLTGSSYDYWGQGTTLTVSS

SEQ ID NO: 36 - protein, 107 aa, synthetic construct
  REGION 1..107: note = 900792-VL
DIQMTQSPASLSASVGESVTITCRASENIYSNLVWYQQKQGKSPQLLVYGARNLADGVPSRFSGSGSGTQFSLKINSLQPEDFGNYYCQHFYETPLTFGTGTKLEIK

SEQ ID NO: 37 - protein, 107 aa, synthetic construct
  REGION 1..107: note = 900792-VL1
DIQMTQSPSSLSASVGDRVTITCRASENIYSNLVWYQQKPGKAPQLLVYGARNLADGVPSRFSGSGSGTQFSLTISSLQPEDFATYYCQHFYETPLTFGTGTKLEIK

SEQ ID NO: 38 - protein, 107 aa, synthetic construct
  REGION 1..107: note = 900792-VL2
DIQMTQSPSSLSASVGDRVTITCRASENIYSNLVWYQQKPGKAPQLLVYGARNLQSGVPSRFSGSGSGTQFSLTISSLQPEDFATYYCQHFYETPLTFGTGTKLEIK

SEQ ID NO: 39 - protein, 107 aa, synthetic construct
  REGION 1..107: note = 900792-VL3
DIQMTQSPSSLSASVGDRVTITCRASENIYSNLVWYQQKPGKAPQLLIYGARNLQSGVPSRFSGSGSGTQFTLTISSLQPEDFATYYCQHFYETPLTFGTGTKLEIK

SEQ ID NO: 40 - protein, 448 aa, synthetic construct
  REGION 1..448: note = 900792 chimeric antibody -VH
QVQLQQSGAELVRPGTSVKVSCKASGYAFTNYLIEWVKQRPGQGLEWIGVINPESGDTYYSEKFKGKATLTADKSSSTAYMQLSSLTSEDSAVYFCAKESLTGSSYDYWGQGTTLTVSSASTKGPSVFPLAPSSKSTSGGTAALGCLVKDYFPEPVTVSWNSGALTSGVHTFPAVLQSSGLYSLSSVVTVPSSSLGTQTYICNVNHKPSNTKVDKRVEPKSCDKTHTCPPCPAPEAAGGPSVFLFPPKPKDTLMISRTPEVTCVVVDVSHEDPEVKFNWYVDGVEVHNAKTKPREEQYNSTYRVVSVLTVLHQDWLNGKEYKCKVSNKALPAPIEKTISKAKGQPREPQVYTLPPSREEMTKNQVSLTCLVKGFYPSDIAVEWESNGQPENNYKTTPPVLDSDGSFFLYSKLTVDKSRWQQGNVFSCSVMHEALHNHYTQKSLSLSPG

SEQ ID NO: 41 - protein, 214 aa, synthetic construct
  REGION 1..214: note = 900792 chimeric antibody -VL
DIQMTQSPASLSASVGESVTITCRASENIYSNLVWYQQKQGKSPQLLVYGARNLADGVPSRFSGSGSGTQFSLKINSLQPEDFGNYYCQHFYETPLTFGTGTKLEIKRTVAAPSVFIFPPSDEQLKSGTASVVCLLNNFYPREAKVQWKVDNALQSGNSQESVTEQDSKDSTYSLSSTLTLSKADYEKHKVYACEVTHQGLSSPVTKSFNRGEC

SEQ ID NO: 42 - protein, 448 aa, synthetic construct
  REGION 1..448: note = 900792-huH1
QVQLQQSGAEVKKPGASVKVSCKASGYAFTNYLIEWVRQAPGQGLEWIGVINPESGDTYYSEKFQGRVTLTADKSTSTAYMELSSLRSEDSAVYFCAKESLTGSSYDYWGQGTTLTVSSASTKGPSVFPLAPSSKSTSGGTAALGCLVKDYFPEPVTVSWNSGALTSGVHTFPAVLQSSGLYSLSSVVTVPSSSLGTQTYICNVNHKPSNTKVDKRVEPKSCDKTHTCPPCPAPEAAGGPSVFLFPPKPKDTLMISRTPEVTCVVVDVSHEDPEVKFNWYVDGVEVHNAKTKPREEQYNSTYRVVSVLTVLHQDWLNGKEYKCKVSNKALPAPIEKTISKAKGQPREPQVYTLPPSREEMTKNQVSLTCLVKGFYPSDIAVEWESNGQPENNYKTTPPVLDSDGSFFLYSKLTVDKSRWQQGNVFSCSVMHEALHNHYTQKSLSLSPG

SEQ ID NO: 43 - protein, 448 aa, synthetic construct
  REGION 1..448: note = 900792-huH2
QVQLVQSGAEVKKPGASVKVSCKASGYAFTNYLIEWVRQAPGQGLEWMGIINPESGDTYYAQKFQGRVTMTADKSTSTAYMELSSLRSEDSAVYFCAKESLTGSSYDYWGQGTTLTVSSASTKGPSVFPLAPSSKSTSGGTAALGCLVKDYFPEPVTVSWNSGALTSGVHTFPAVLQSSGLYSLSSVVTVPSSSLGTQTYICNVNHKPSNTKVDKRVEPKSCDKTHTCPPCPAPEAAGGPSVFLFPPKPKDTLMISRTPEVTCVVVDVSHEDPEVKFNWYVDGVEVHNAKTKPREEQYNSTYRVVSVLTVLHQDWLNGKEYKCKVSNKALPAPIEKTISKAKGQPREPQVYTLPPSREEMTKNQVSLTCLVKGFYPSDIAVEWESNGQPENNYKTTPPVLDSDGSFFLYSKLTVDKSRWQQGNVFSCSVMHEALHNHYTQKSLSLSPG

SEQ ID NO: 44 - protein, 448 aa, synthetic construct
  REGION 1..448: note = 900792-huH3
QVQLQQSGAEVKKPGASVKVSCKASGYAFTNYLIEWVRQAPGQGLEWMGVINPESGDTYYSQKFQGRVTMTADKSTSTAYMELSSLRSEDSAVYFCAKESLTGSSYDYWGQGTTLTVSSASTKGPSVFPLAPSSKSTSGGTAALGCLVKDYFPEPVTVSWNSGALTSGVHTFPAVLQSSGLYSLSSVVTVPSSSLGTQTYICNVNHKPSNTKVDKRVEPKSCDKTHTCPPCPAPEAAGGPSVFLFPPKPKDTLMISRTPEVTCVVVDVSHEDPEVKFNWYVDGVEVHNAKTKPREEQYNSTYRVVSVLTVLHQDWLNGKEYKCKVSNKALPAPIEKTISKAKGQPREPQVYTLPPSREEMTKNQVSLTCLVKGFYPSDIAVEWESNGQPENNYKTTPPVLDSDGSFFLYSKLTVDKSRWQQGNVFSCSVMHEALHNHYTQKSLSLSPG

SEQ ID NO: 45 - protein, 448 aa, synthetic construct
  REGION 1..448: note = 900792-huH4
QVQLVQSGAEVKKPGASVKVSCKASGYAFTNYLIEWVRQAPGQGLEWMGIINPESGDTYYAQKFQGRVTLTADKSTSTAYMELSSLRSEDSAVYYCAKESLTGSSYDYWGQGTTLTVSSASTKGPSVFPLAPSSKSTSGGTAALGCLVKDYFPEPVTVSWNSGALTSGVHTFPAVLQSSGLYSLSSVVTVPSSSLGTQTYICNVNHKPSNTKVDKRVEPKSCDKTHTCPPCPAPEAAGGPSVFLFPPKPKDTLMISRTPEVTCVVVDVSHEDPEVKFNWYVDGVEVHNAKTKPREEQYNSTYRVVSVLTVLHQDWLNGKEYKCKVSNKALPAPIEKTISKAKGQPREPQVYTLPPSREEMTKNQVSLTCLVKGFYPSDIAVEWESNGQPENNYKTTPPVLDSDGSFFLYSKLTVDKSRWQQGNVFSCSVMHEALHNHYTQKSLSLSPG

SEQ ID NO: 46 - protein, 214 aa, synthetic construct
  REGION 1..214: note = 900792-huL1
DIQMTQSPSSLSASVGDRVTITCRASENIYSNLVWYQQKPGKAPQLLVYGARNLADGVPSRFSGSGSGTQFSLTISSLQPEDFATYYCQHFYETPLTFGTGTKLEIKRTVAAPSVFIFPPSDEQLKSGTASVVCLLNNFYPREAKVQWKVDNALQSGNSQESVTEQDSKDSTYSLSSTLTLSKADYEKHKVYACEVTHQGLSSPVTKSFNRGEC

SEQ ID NO: 47 - protein, 214 aa, synthetic construct
  REGION 1..214: note = 900792-huL2
DIQMTQSPSSLSASVGDRVTITCRASENIYSNLVWYQQKPGKAPQLLVYGARNLQSGVPSRFSGSGSGTQFSLTISSLQPEDFATYYCQHFYETPLTFGTGTKLEIKRTVAAPSVFIFPPSDEQLKSGTASVVCLLNNFYPREAKVQWKVDNALQSGNSQESVTEQDSKDSTYSLSSTLTLSKADYEKHKVYACEVTHQGLSSPVTKSFNRGEC

SEQ ID NO: 48 - protein, 214 aa, synthetic construct
  REGION 1..214: note = 900792-huL3
DIQMTQSPSSLSASVGDRVTITCRASENIYSNLVWYQQKPGKAPQLLIYGARNLQSGVPSRFSGSGSGTQFTLTISSLQPEDFATYYCQHFYETPLTFGTGTKLEIKRTVAAPSVFIFPPSDEQLKSGTASVVCLLNNFYPREAKVQWKVDNALQSGNSQESVTEQDSKDSTYSLSSTLTLSKADYEKHKVYACEVTHQGLSSPVTKSFNRGEC